European Patent Specification EP 3 534 932 B1, published May 22, 2024. Title: TREATMENT OF DISEASES RELATED TO IGFB3 AND ITS RECEPTOR. Applicant: Virginia Commonwealth University Oh, Youngman Doxmorov, Mikhail Cai, Qing. The sequence listing filed with the application follows.

SEQUENCE LISTING (33 sequences)

SEQ ID NO: 1 - DNA, 352 bp, Artificial Sequence
  Synthetic antibody
cagatccagttggtgcagtctggacctgagctgaaggagcctggagagacagtcaagatctcctgcaaggcttctgggtatactttcacaaactatggaatgaactgggtgaagcaggctccaggaagggtttaaagtggatgggctggataaacacctacaccagagagacaacatatattgatgagttcaagggacggtctgccttctctatggaaacctctgccagcactgcctatttgcagatctacaactcaaaaatgaggacacggctacatatttctgtgcaagagggtctacgatgtatggtctggacaagtggggtcaaggaacctcagtcaccgtctcctca

SEQ ID NO: 2 - protein, 118 aa, Artificial Sequence
  Synthetic antibody
QIQLVQSGPELKEPGETVKISCKASGYTFTNYGMNWVKQAPGKGLKWMGWINTYTRETTYIDEFKGRSAFSMETSASTAYLQIYNLKNEDTATYFCARGSTMYGLDKWGQGTSVTVSS

SEQ ID NO: 3 - DNA, 322 bp, Artificial Sequence
  Synthetic antibody
gacattgtgatgacccagtctcaaaaattcatgtccacatcagtgggagacggggtcagcgtcacctgtaaggccagtcagaatgtgggtactaatgtagtctggtatcaacagaaaccagggcaattcctaaggcactgatttactcggcatcctaccggtacagtggagtccctgatcgcttcacaggcagtggatctgggacagatttcactctcaccatcagcaatgtgcagtctgaagacttggcagaaatttctgtcaccaatataacagctatcctctcacgttcggtgctgggaccaagctggagctgaaacgg

SEQ ID NO: 4 - protein, 108 aa, Artificial Sequence
  Synthetic antibody
DIVMTQSQKFMSTSVGDGVSVTCKASQNVGTNVVWYQQKPGQSPKALIYSASYRYSGVPDRFTGSGSGTDFTLTISNVQSEDLAEYFCHQYNSYPLTFGAGTKLELKR

SEQ ID NO: 5 - DNA, 354 bp, Artificial Sequence
  Synthetic antibody
cagatccagttggtgcagtctggacctgagctgaaggagcctggagagacagtcaagatctcctgcaaggcttctgggtatactttcacaaactatggaatgaactgggtgaagcaggctccaggaaagggtttaaagtggatgggctggataaacacctacaccagagagacaacatatattgatgagttcaagggacggtctgccttctctatggaaacctctgccagcactgcctatttgcagatctacaacctcaaaaatgaggacacggctacatatttctgtgcaagagggtctacgatgtatggtctggacaagtggggtcaaggaacctcagtcaccgtctcctca

SEQ ID NO: 6 - protein, 118 aa, Artificial Sequence; identical to SEQ ID NO: 2
  Synthetic antibody

SEQ ID NO: 7 - DNA, 324 bp, Artificial Sequence
  Synthetic antibody
gacattgtgatgacccagtctcaaaaattcatgtccacatcagtgggagacggggtcagcgtcacctgtaaggccagtcagaatgtgggtactaatgtagtctggtatcaacagaaaccagggcaatctcctaaggcactgatttactcggcatcctaccggtacagtggagtccctgatcgcttcacaggcagtggatctgggacagatttcactctcaccatcagcaatgtgcagtctgaagacttggcagaatatttctgtcaccaatataacagctatcctctcacgttcggtgctgggaccaagctggagctgaaacgg

SEQ ID NO: 8 - protein, 108 aa, Artificial Sequence; identical to SEQ ID NO: 4
  Synthetic antibody

SEQ ID NO: 9 - DNA, 1419 bp, Artificial Sequence
  Synthetic antibody
atggaccccaagggcagcctgagctggagaatcctgctgttcctgagcctggccttcgagctgagctacggccagatccagttggtgcagtctggacctgagctgaaggagcctggagagacagtcaagatctcctgcaaggcttctgggtatactttcacaaactatggaatgaactgggtgaagcaggctccaggaaagggtttaaagtggatgggctggataaacacctacaccagagagacaacatatattgatgagttcaagggacggtctgccttctctatggaaacctctgccagcactgcctatttgcagatctacaacctcaaaaatgaggacacggctacatatttctgtgcaagagggtctacgatgtatggtctggacaagtggggtcaaggaacctcagtcaccgtctcctcagctagcaccaagggccccagcgtgttccctctggcccccagcagcaagagcaccagcggcggaaccgccgccctgggctgcctggtgaaggactacttccccgagcccgtgaccgtgtcctggaacagcggcgctctgaccagcggagtgcacaccttccctgccgtgctgcagagcagcggcctgtactccctgagcagcgtggtgaccgtgcccagcagcagcctgggcacccagacctacatctgcaacgtgaaccacaagccctccaacaccaaggtggacaagaaggtggagcctaagagctgcgacaagacccacacctgccctccctgccccgcccccgagctgctgggcggacccagcgtgttcctgttccctcccaagcccaaggacaccctgatgatcagccgcacccccgaggtgacctgcgtggtggtggacgtgagccacgaggaccccgaggtgaagttcaactggtacgtggacggcgtggaggtgcacaacgccaagaccaagcctcgggaggagcagtacaactccacctaccgcgtggtgagcgtgctgaccgtgctgcaccaggactggctgaacggcaaggagtacaagtgcaaggtgagcaacaaggccctgcccgctcccatcgagaagaccatcagcaaggccaagggccagccccgggagcctcaggtgtacaccctgccccccagccgcgacgagctgaccaagaaccaggtgagcctgacctgcctggtgaagggcttctacccctccgacatcgccgtggagtgggagagcaacggccagcctgagaacaactacaagaccacccctcccgtgctggacagcgacggcagcttcttcctgtacagcaagctgaccgtggacaagtcccggtggcagcagggcaacgtgttcagctgcagcgtgatgcacgaggccctgcacaaccactacacccagaagagcctgagcctgagccccggatagtaa

SEQ ID NO: 10 - protein, 471 aa, Artificial Sequence
  Synthetic antibody
MDPKGSLSWRILLFLSLAFELSYGQIQLVQSGPELKEPGETVKISCKASGYTFTNYGMNWVKQAPGKGLKWMGWINTYTRETTYIDEFKGRSAFSMETSASTAYLQIYNLKNEDTATYFCARGSTMYGLDKWGQGTSVTVSSASTKGPSVFPLAPSSKSTSGGTAALGCLVKDYFPEPVTVSWNSGALTSGVHTFPAVLQSSGLYSLSSVVTVPSSSLGTQTYICNVNHKPSNTKVDKKVEPKSCDKTHTCPPCPAPELLGGPSVFLFPPKPKDTLMISRTPEVTCVVVDVSHEDPEVKFNWYVDGVEVHNAKTKPREEQYNSTYRVVSVLTVLHQDWLNGKEYKCKVSNKALPAPIEKTISKAKGQPREPQVYTLPPSRDELTKNQVSLTCLVKGFYPSDIAVEWESNGQPENNYKTTPPVLDSDGSFFLYSKLTVDKSRWQQGNVFSCSVMHEALHNHYTQKSLSLSPG

SEQ ID NO: 11 - DNA, 705 bp, Artificial Sequence
  Synthetic antibody
atggagaccgacaccctgctgctctgggtgctgctgctctgggtgcccggctccaccggagacattgtgatgacccagtctcaaaaattcatgtccacatcagtgggagacggggtcagcgtcacctgtaaggccagtcagaatgtgggtactaatgtagtctggtatcaacagaaaccagggcaatctcctaaggcactgatttactcggcatcctaccggtacagtggagtccctgatcgcttcacaggcagtggatctgggacagatttcactctcaccatcagcaatgtgcagtctgaagacttggcagaatatttctgtcaccaatataacagctatcctctcacgttcggtgctgggaccaagctggagctgaaacggaccgtggccgcccccagcgtgttcatcttccctcccagcgacgagcagctgaagtctggcaccgccagcgtggtgtgcctgctgaacaacttctacccccgcgaggccaaggtgcagtggaaggtggacaacgccctgcagagcggcaacagccaggagagcgtgaccgagcaggactccaaggacagcacctacagcctgagcagcaccctgaccctgagcaaggccgactacgagaagcacaaggtgtacgcctgcgaggtgacccaccagggactgtctagccccgtgaccaagagcttcaaccggggcgagtgctaa

SEQ ID NO: 12 - protein, 234 aa, Artificial Sequence
  Synthetic antibody
METDTLLLWVLLLWVPGSTGDIVMTQSQKFMSTSVGDGVSVTCKASQNVGTNVVWYQQKPGQSPKALIYSASYRYSGVPDRFTGSGSGTDFTLTISNVQSEDLAEYFCHQYNSYPLTFGAGTKLELKRTVAAPSVFIFPPSDEQLKSGTASVVCLLNNFYPREAKVQWKVDNALQSGNSQESVTEQDSKDSTYSLSSTLTLSKADYEKHKVYACEVTHQGLSSPVTKSFNRGEC

SEQ ID NO: 13 - protein, 10 aa, Artificial Sequence
  Synthetic peptide
GLKGSSAGQL

SEQ ID NO: 14 - DNA, 24 bp, Artificial Sequence
  Synthetic CDR sequence
gggtttaccttcacatactatgga

SEQ ID NO: 15 - protein, 8 aa, Artificial Sequence
  Synthetic CDR sequence
GFTFTYYG

SEQ ID NO: 16 - DNA, 24 bp, Artificial Sequence
  Synthetic CDR sequence
ataaacacctacactggagagcca

SEQ ID NO: 17 - protein, 8 aa, Artificial Sequence
  Synthetic CDR sequence
INTYTGEP

SEQ ID NO: 18 - DNA, 33 bp, Artificial Sequence
  Synthetic CDR sequence
gcaagagggcgtacggtagtgggctttgactct

SEQ ID NO: 19 - protein, 11 aa, Artificial Sequence
  Synthetic CDR sequence
ARGRTVVGFDS

SEQ ID NO: 20 - DNA, 18 bp, Artificial Sequence
  Synthetic CDR sequence
caggacattggtagtagc

SEQ ID NO: 21 - protein, 6 aa, Artificial Sequence
  Synthetic CDR sequence
QDIGSS

SEQ ID NO: 22 - DNA, 27 bp, Artificial Sequence
  Synthetic CDR sequence
ctacaatatgctagttctccgtacacg

SEQ ID NO: 23 - protein, 7 aa, Artificial Sequence
  Synhetic CDR sequence
LQYASSP

SEQ ID NO: 24 - DNA, 24 bp, Artificial Sequence
  Synthetic CDR sequence
gggtatactttcacaaactatgga

SEQ ID NO: 25 - protein, 8 aa, Artificial Sequence
  Synthetic CDR sequence
GYTFTNYG

SEQ ID NO: 26 - DNA, 24 bp, Artificial Sequence
  Syntehtic CDR sequence
ataaacacctacaccagagagaca

SEQ ID NO: 27 - protein, 8 aa, Artificial Sequence
  Synthetic CDR sequence
INTYTRET

SEQ ID NO: 28 - DNA, 33 bp, Artificial Sequence
  Synthetic CDR sequence
gcaagagggtctacgatgtatggtctggacaag

SEQ ID NO: 29 - protein, 11 aa, Artificial Sequence
  Synthetic CDR sequence
ARGSTMYGLDK

SEQ ID NO: 30 - DNA, 18 bp, Artificial Sequence
  Synthetic CDR sequence
cagaatgtgggtactaat

SEQ ID NO: 31 - protein, 6 aa, Artificial Sequence
  Synthetic CDR sequence
QNVGTN

SEQ ID NO: 32 - DNA, 27 bp, Artificial Sequence
  Synthetic CDR sequence
caccaatataacagctatcctctcacg

SEQ ID NO: 33 - protein, 9 aa, Artificial Sequence
  Synthetic CDR sequence
HQYNSYPLT